European Patent Application EP 4 748 926 A1, published May 27, 2026. Title: 프럭토키나제 변이체 및 이를 이용한 L-아미노산 생산 방법. Applicant: 씨제이제일제당 주식회사. The sequence listing filed with the application follows.

SEQUENCE LISTING (85 sequences)

SEQ ID NO: 1 - protein, 304 aa, Echerichia coli
MSAKVWVLGDAVVDLLPESDGRLLPCPGGAPANVAVGIARLGGTSGFIGRVGDDPFGALMQRTLLTEGVDITYLKQDEWHRTSTVLVDLNDQGERSFTFMVRPSADLFLETTDLPCWRHGEWLHLCSIALSAEPSRTSAFTAMTAIRHAGGFVSFDPNIREDLWQDEHLLRLCLRQALQLADVVKLSEEEWRLISGKTQNDQDICALAKEYEIAMLLVTKGAEGVVVCYRGQVHHFAGMSVNCVDSTGAGDAFVAGLLTGLSSTGLSTDEREMRRIIDLAQRCGALAVTAKGAMTALPCRQELE

SEQ ID NO: 2 - DNA, 915 bp, Echerichia coli
  source 1..915: mol_type = other DNA
atgtcagccaaagtatgggttttaggggatgcggtcgtagatctcttgccagaatcagacgggcgcctactgccttgtcctggcggcgcgccagctaacgttgcggtgggaatcgccagattaggcggaacaagtgggtttataggtcgggtgggggatgatccttttggtgcgttaatgcaaagaacgctgctaactgagggagtcgatatcacgtatctgaagcaagatgaatggcaccggacatccacggtgcttgtcgatctgaacgatcaaggggaacgttcatttacgtttatggtccgccccagtgccgatctttttttagagacgacagacttgccctgctggcgacatggcgaatggttacatctctgttcaattgcgttgtctgccgagccttcgcgtaccagcgcatttactgcgatgacggcgatccggcatgccggaggttttgtcagcttcgatcctaatattcgtgaagatctatggcaagacgagcatttgctccgcttgtgtttgcggcaggcgctacaactggcggatgtcgtcaagctctcggaagaagaatggcgacttatcagtggaaaaacacagaacgatcaggatatatgcgccctggcaaaagagtatgagatcgccatgctgttggtgactaaaggtgcagaaggggtggtggtctgttatcgaggacaagttcaccattttgctggaatgtctgtgaattgtgtcgatagcacgggggcgggagatgcgttcgttgccgggttactcacaggtctgtcctctacgggattatctacagatgagagagaaatgcgacgaattatcgatctcgctcaacgttgcggagcgcttgcagtaacggcgaaaggggcaatgacagcgctgccatgtcgacaagaactggaatag

SEQ ID NO: 3 - protein, 304 aa, synthetic construct
MSAKVWVLGDAVVDLLPESDGRLLPCPGGAPANVAVGIARLGGTSGFIGRVGDDPFGALMQRTLLTEGVDITYLKQDECHRTSTVLVDLNDQGERSFTFMVRPSADLFLETTDLPCWRHGEWLHLCSIALSAEPSRTSAFTAMTAIRHAGGFVSFDPNIREDLWQDEHLLRLCLRQALQLADVVKLSEEEWRLISGKTQNDQDICALAKEYEIAMLLVTKGAEGVVVCYRGQVHHFAGMSVNCVDSTGAGDAFVAGLLTGLSSTGLSTDEREMRRIIDLAQRCGALAVTAKGAMTALPCRQELE

SEQ ID NO: 4 - DNA, 915 bp, synthetic construct
  source 1..915: mol_type = other DNA
atgtcagccaaagtatgggttttaggggatgcggtcgtagatctcttgccagaatcagacgggcgcctactgccttgtcctggcggcgcgccagctaacgttgcggtgggaatcgccagattaggcggaacaagtgggtttataggtcgggtgggggatgatccttttggtgcgttaatgcaaagaacgctgctaactgagggagtcgatatcacgtatctgaagcaagatgaatgtcaccggacatccacggtgcttgtcgatctgaacgatcaaggggaacgttcatttacgtttatggtccgccccagtgccgatctttttttagagacgacagacttgccctgctggcgacatggcgaatggttacatctctgttcaattgcgttgtctgccgagccttcgcgtaccagcgcatttactgcgatgacggcgatccggcatgccggaggttttgtcagcttcgatcctaatattcgtgaagatctatggcaagacgagcatttgctccgcttgtgtttgcggcaggcgctacaactggcggatgtcgtcaagctctcggaagaagaatggcgacttatcagtggaaaaacacagaacgatcaggatatatgcgccctggcaaaagagtatgagatcgccatgctgttggtgactaaaggtgcagaaggggtggtggtctgttatcgaggacaagttcaccattttgctggaatgtctgtgaattgtgtcgatagcacgggggcgggagatgcgttcgttgccgggttactcacaggtctgtcctctacgggattatctacagatgagagagaaatgcgacgaattatcgatctcgctcaacgttgcggagcgcttgcagtaacggcgaaaggggcaatgacagcgctgccatgtcgacaagaactggaatag

SEQ ID NO: 5 - protein, 304 aa, synthetic construct
MSAKVWVLGDAVVDLLPESDGRLLPCPGGAPANVAVGIARLGGTSGFIGRVGDDPFGALMQRTLLTEGVDITYLKQDEWHRTSTVLVDLNDQGERSFTFMVRPSADLFLETTDLPCWRHGEWLHLCSIALSAEPSRTSAFTAMTAIRHAGGFVSFDPNIREDLWQDEHLLRLCLRQALQLVDVVKLSEEEWRLISGKTQNDQDICALAKEYEIAMLLVTKGAEGVVVCYRGQVHHFAGMSVNCVDSTGAGDAFVAGLLTGLSSTGLSTDEREMRRIIDLAQRCGALAVTAKGAMTALPCRQELE

SEQ ID NO: 6 - DNA, 915 bp, synthetic construct
  source 1..915: mol_type = other DNA
atgtcagccaaagtatgggttttaggggatgcggtcgtagatctcttgccagaatcagacgggcgcctactgccttgtcctggcggcgcgccagctaacgttgcggtgggaatcgccagattaggcggaacaagtgggtttataggtcgggtgggggatgatccttttggtgcgttaatgcaaagaacgctgctaactgagggagtcgatatcacgtatctgaagcaagatgaatggcaccggacatccacggtgcttgtcgatctgaacgatcaaggggaacgttcatttacgtttatggtccgccccagtgccgatctttttttagagacgacagacttgccctgctggcgacatggcgaatggttacatctctgttcaattgcgttgtctgccgagccttcgcgtaccagcgcatttactgcgatgacggcgatccggcatgccggaggttttgtcagcttcgatcctaatattcgtgaagatctatggcaagacgagcatttgctccgcttgtgtttgcggcaggcgctacaactggtggatgtcgtcaagctctcggaagaagaatggcgacttatcagtggaaaaacacagaacgatcaggatatatgcgccctggcaaaagagtatgagatcgccatgctgttggtgactaaaggtgcagaaggggtggtggtctgttatcgaggacaagttcaccattttgctggaatgtctgtgaattgtgtcgatagcacgggggcgggagatgcgttcgttgccgggttactcacaggtctgtcctctacgggattatctacagatgagagagaaatgcgacgaattatcgatctcgctcaacgttgcggagcgcttgcagtaacggcgaaaggggcaatgacagcgctgccatgtcgacaagaactggaatag

SEQ ID NO: 7 - protein, 304 aa, synthetic construct
MSAKVWVLGDAVVDLLPESDGRLLPCPGGAPANVAVGIARLGGTSGFIGRVGDDPFGALMQRTLLTEGVDITYLKQDECHRTSTVLVDLNDQGERSFTFMVRPSADLFLETTDLPCWRHGEWLHLCSIALSAEPSRTSAFTAMTAIRHAGGFVSFDPNIREDLWQDEHLLRLCLRQALQLVDVVKLSEEEWRLISGKTQNDQDICALAKEYEIAMLLVTKGAEGVVVCYRGQVHHFAGMSVNCVDSTGAGDAFVAGLLTGLSSTGLSTDEREMRRIIDLAQRCGALAVTAKGAMTALPCRQELE

SEQ ID NO: 8 - DNA, 915 bp, synthetic construct
  source 1..915: mol_type = other DNA
atgtcagccaaagtatgggttttaggggatgcggtcgtagatctcttgccagaatcagacgggcgcctactgccttgtcctggcggcgcgccagctaacgttgcggtgggaatcgccagattaggcggaacaagtgggtttataggtcgggtgggggatgatccttttggtgcgttaatgcaaagaacgctgctaactgagggagtcgatatcacgtatctgaagcaagatgaatgtcaccggacatccacggtgcttgtcgatctgaacgatcaaggggaacgttcatttacgtttatggtccgccccagtgccgatctttttttagagacgacagacttgccctgctggcgacatggcgaatggttacatctctgttcaattgcgttgtctgccgagccttcgcgtaccagcgcatttactgcgatgacggcgatccggcatgccggaggttttgtcagcttcgatcctaatattcgtgaagatctatggcaagacgagcatttgctccgcttgtgtttgcggcaggcgctacaactggtggatgtcgtcaagctctcggaagaagaatggcgacttatcagtggaaaaacacagaacgatcaggatatatgcgccctggcaaaagagtatgagatcgccatgctgttggtgactaaaggtgcagaaggggtggtggtctgttatcgaggacaagttcaccattttgctggaatgtctgtgaattgtgtcgatagcacgggggcgggagatgcgttcgttgccgggttactcacaggtctgtcctctacgggattatctacagatgagagagaaatgcgacgaattatcgatctcgctcaacgttgcggagcgcttgcagtaacggcgaaaggggcaatgacagcgctgccatgtcgacaagaactggaatag

SEQ ID NO: 9 - DNA, 36 bp, synthetic construct
  source 1..36: mol_type = other DNA
ttcgagctcggtaccccaaatgctccaaccgtccgt

SEQ ID NO: 10 - DNA, 33 bp, synthetic construct
  source 1..33: mol_type = other DNA
cgctgggatgtttctgaactcattccttctgct

SEQ ID NO: 11 - DNA, 34 bp, synthetic construct
  source 1..34: mol_type = other DNA
acaagaactggaataggacatctaataaccgggc

SEQ ID NO: 12 - DNA, 34 bp, synthetic construct
  source 1..34: mol_type = other DNA
ctctagaggatcccctacacctccacctgcccag

SEQ ID NO: 13 - DNA, 40 bp, synthetic construct
  source 1..40: mol_type = other DNA
cccaacgaaaggaaacactcatgtcagccaaagtatgggt

SEQ ID NO: 14 - DNA, 36 bp, synthetic construct
  source 1..36: mol_type = other DNA
tgcccggttattagatgtcctattccagttcttgtc

SEQ ID NO: 15 - DNA, 23 bp, synthetic construct
  source 1..23: mol_type = other DNA
atgtccggtgacattcatcttgc

SEQ ID NO: 16 - DNA, 23 bp, synthetic construct
  source 1..23: mol_type = other DNA
aagatgaatgtcaccggacatcc

SEQ ID NO: 17 - DNA, 30 bp, synthetic construct
  source 1..30: mol_type = other DNA
acatccaccagttgtagcgcctgccgcaaa

SEQ ID NO: 18 - DNA, 30 bp, synthetic construct
  source 1..30: mol_type = other DNA
aactggtggatgtcgtcaagctctcggaag

SEQ ID NO: 19 - DNA, 318 bp, synthetic construct
  source 1..318: mol_type = other DNA
agaaacatcccagcgctactaatagggagcgttgaccttccttccacggaccggtaatcggagtgcctaaaaccgcatgcggcttaggctccaagataggttctgcgcggccgggtaatgcatcttctttagcaacaagttgaggggtaggtgcaaataagaacgacatagaaatcgtctcctttctgtttttaatcaacatacaccaccacctaaaaattccccgaccagcaagttcacagtattcgggcacaatatcgttgccaaaatattgtttcggaatatcatgggatacgtacccaacgaaaggaaacactc

SEQ ID NO: 20 - DNA, 37 bp, synthetic construct
  source 1..37: mol_type = other DNA
gcagaaggaatgagttcagaaacatcccagcgctact

SEQ ID NO: 21 - DNA, 36 bp, synthetic construct
  source 1..36: mol_type = other DNA
tactttggctgacatgagtgtttcctttcgttgggt

SEQ ID NO: 22 - protein, 281 aa, synthetic construct
MLKIAVPNKGSLSERAMEILAEAGYAGRGDSKSLNVFDEANNVEFFFLRPKDIAIYVAGGQLDLGITGRDLARDSQADVHEVLSLGFGSSTFRYAAPADEEWSIEKLDGKRIATSYPNLVRDDLAARGLSAEVLRLDGAVEVSIKLGVADAIADVVSTGRTLRQQGLAPFGEVLCTSEAVIVGRKDEKVTPEQQILLRRIQGILHAQNFLMLDYNVDRDNLDAATAVTPGLSHPQVSPLARDNWVAVRAMVPRRSANAIMDKLAGLGAEAILASEIRIARI

SEQ ID NO: 23 - DNA, 30 bp, synthetic construct
  source 1..30: mol_type = other DNA
gaggagatcaaaacaatgaagacatttgac

SEQ ID NO: 24 - DNA, 30 bp, synthetic construct
  source 1..30: mol_type = other DNA
acaccaagcttgatggatacctctactgca

SEQ ID NO: 25 - DNA, 29 bp, synthetic construct
  source 1..29: mol_type = other DNA
cagtagaggtatccatcaagcttggtgtc

SEQ ID NO: 26 - DNA, 28 bp, synthetic construct
  source 1..28: mol_type = other DNA
actctagaggatccccctagatgcgggc

SEQ ID NO: 27 - DNA, 34 bp, synthetic construct
  source 1..34: mol_type = other DNA
tcgagctcggtacccaccgaactcctgacagagt

SEQ ID NO: 28 - DNA, 30 bp, synthetic construct
  source 1..30: mol_type = other DNA
acatgaagcgcctcggtacattcttccaca

SEQ ID NO: 29 - DNA, 294 bp, synthetic construct
  source 1..294: mol_type = other DNA
ggcgcttcatgtcaacaatctttaacgttttcaagttcacaagtcgtgttcaaatggtgacaagattggacactgtgctgaattggcaccaagccctcataaatgatagatctaaatcgaatatcaatatatggtctgtttattggaacgcgtcccagtggctgagacgcatccgctaaagccccaggaaccctgtgcagaaagaacaaataatcgtgaattttggcagcaacagcggggcctggtataattgaaaacgtgcaaaagcatagattattggaggagatcaaaaca

SEQ ID NO: 30 - DNA, 30 bp, synthetic construct
  source 1..30: mol_type = other DNA
aagaatgtaccgaggcgcttcatgtcaaca

SEQ ID NO: 31 - DNA, 30 bp, synthetic construct
  source 1..30: mol_type = other DNA
caaatgtcttcattgttttgatctcctcca

SEQ ID NO: 32 - DNA, 19 bp, synthetic construct
  source 1..19: mol_type = other DNA
actgcctggtaccaccaga

SEQ ID NO: 33 - DNA, 20 bp, synthetic construct
  source 1..20: mol_type = other DNA
ctgcctctcacaagttgaag

SEQ ID NO: 34 - DNA, 30 bp, synthetic construct
  source 1..30: mol_type = other DNA
tcgagctcggtacccattggtgctcggcgc

SEQ ID NO: 35 - DNA, 29 bp, synthetic construct
  source 1..29: mol_type = other DNA
tgggatgtttctgtgttgttagtctagtg

SEQ ID NO: 36 - DNA, 34 bp, synthetic construct
  source 1..34: mol_type = other DNA
tcgagctcggtacccaaccaagtttagatgcgcc

SEQ ID NO: 37 - DNA, 31 bp, synthetic construct
  source 1..31: mol_type = other DNA
gctgggatgtttctgccgatagtttatgtca

SEQ ID NO: 38 - DNA, 35 bp, synthetic construct
  source 1..35: mol_type = other DNA
tcgagctcggtacccggtgacagctcgcgccgcat

SEQ ID NO: 39 - DNA, 32 bp, synthetic construct
  source 1..32: mol_type = other DNA
gcgctgggatgtttctggcgaaaagttctccc

SEQ ID NO: 40 - DNA, 33 bp, synthetic construct
  source 1..33: mol_type = other DNA
tcgagctcggtacccttgatgcctgcatgaagg

SEQ ID NO: 41 - DNA, 31 bp, synthetic construct
  source 1..31: mol_type = other DNA
tgacatgaagcgccgaatattgatcctatct

SEQ ID NO: 42 - DNA, 33 bp, synthetic construct
  source 1..33: mol_type = other DNA
ttcgagctcggtacccaccttcagcaaccactc

SEQ ID NO: 43 - DNA, 29 bp, synthetic construct
  source 1..29: mol_type = other DNA
tgacatgaagcgccgaaaaattcttctct

SEQ ID NO: 44 - DNA, 32 bp, synthetic construct
  source 1..32: mol_type = other DNA
aaaggaaacactcatgagcaaatatgcagacg

SEQ ID NO: 45 - DNA, 27 bp, synthetic construct
  source 1..27: mol_type = other DNA
ctagaggatcccccagccggagaggga

SEQ ID NO: 46 - DNA, 30 bp, synthetic construct
  source 1..30: mol_type = other DNA
aaaggaaacactcatgaccaaaactgtcgc

SEQ ID NO: 47 - DNA, 31 bp, synthetic construct
  source 1..31: mol_type = other DNA
ctagaggatccccacctctggaggcgtggtc

SEQ ID NO: 48 - DNA, 34 bp, synthetic construct
  source 1..34: mol_type = other DNA
cgaaaggaaacactcatgttgaatgtcactgacc

SEQ ID NO: 49 - DNA, 32 bp, synthetic construct
  source 1..32: mol_type = other DNA
ctagaggatccccccgtgctcagcctgaggag

SEQ ID NO: 50 - DNA, 33 bp, synthetic construct
  source 1..33: mol_type = other DNA
ggagatcaaaacaatgaccttcactattcttcc

SEQ ID NO: 51 - DNA, 32 bp, synthetic construct
  source 1..32: mol_type = other DNA
ctagaggatccccacgaaacgtgcacaacctt

SEQ ID NO: 52 - DNA, 27 bp, synthetic construct
  source 1..27: mol_type = other DNA
gagatcaaaacaatgactgtcgcacca

SEQ ID NO: 53 - DNA, 32 bp, synthetic construct
  source 1..32: mol_type = other DNA
ctagaggatccccgggtcgcggccgtagtggc

SEQ ID NO: 54 - DNA, 32 bp, synthetic construct
  source 1..32: mol_type = other DNA
actagactaacaacacagaaacatcccagcgc

SEQ ID NO: 55 - DNA, 30 bp, synthetic construct
  source 1..30: mol_type = other DNA
tctgcatatttgctcatgagtgtttccttt

SEQ ID NO: 56 - DNA, 33 bp, synthetic construct
  source 1..33: mol_type = other DNA
acataaactatcggcagaaacatcccagcgcta

SEQ ID NO: 57 - DNA, 30 bp, synthetic construct
  source 1..30: mol_type = other DNA
gacagttttggtcatgagtgtttcctttcg

SEQ ID NO: 58 - DNA, 31 bp, synthetic construct
  source 1..31: mol_type = other DNA
gagaacttttcgccagaaacatcccagcgct

SEQ ID NO: 59 - DNA, 30 bp, synthetic construct
  source 1..30: mol_type = other DNA
agtgacattcaacatgagtgtttcctttcg

SEQ ID NO: 60 - DNA, 29 bp, synthetic construct
  source 1..29: mol_type = other DNA
aggatcaatattcggcgcttcatgtcaac

SEQ ID NO: 61 - DNA, 30 bp, synthetic construct
  source 1..30: mol_type = other DNA
gaatagtgaaggtcattgttttgatctcct

SEQ ID NO: 62 - DNA, 29 bp, synthetic construct
  source 1..29: mol_type = other DNA
gagaagaatttttcggcgcttcatgtcaa

SEQ ID NO: 63 - DNA, 29 bp, synthetic construct
  source 1..29: mol_type = other DNA
tggtgcgacagtcattgttttgatctcct

SEQ ID NO: 64 - DNA, 15 bp, synthetic construct
  source 1..15: mol_type = other DNA
gagcatgcatcaaag

SEQ ID NO: 65 - DNA, 19 bp, synthetic construct
  source 1..19: mol_type = other DNA
agaaatttgatccttataa

SEQ ID NO: 66 - DNA, 17 bp, synthetic construct
  source 1..17: mol_type = other DNA
ttgagagatgcttatcg

SEQ ID NO: 67 - DNA, 20 bp, synthetic construct
  source 1..20: mol_type = other DNA
cacttcagtgcggattccaa

SEQ ID NO: 68 - DNA, 17 bp, synthetic construct
  source 1..17: mol_type = other DNA
agcgggtttaattcagg

SEQ ID NO: 69 - DNA, 18 bp, synthetic construct
  source 1..18: mol_type = other DNA
gtgggtaagggttttcgt

SEQ ID NO: 70 - DNA, 19 bp, synthetic construct
  source 1..19: mol_type = other DNA
cacgaaaatgatcgttttg

SEQ ID NO: 71 - DNA, 18 bp, synthetic construct
  source 1..18: mol_type = other DNA
tatgggattcgatggcca

SEQ ID NO: 72 - DNA, 19 bp, synthetic construct
  source 1..19: mol_type = other DNA
tgtgggaatcgctgggcac

SEQ ID NO: 73 - DNA, 16 bp, synthetic construct
  source 1..16: mol_type = other DNA
cggtcgcccgcatctg

SEQ ID NO: 74 - DNA, 1311 bp, synthetic construct
  source 1..1311: mol_type = other DNA
atgaagtctaccggcaacatcatcgctgacaccatctgccgcactgcggaactaggactcaccatcaccggcgcttccgatgcaggtgattacaccctgatcgaagcagacgcactcgactacacctccacctgcccagaatgctcccaacctggggtgtttcgtcatcacacccaccggatgctcattgatttacccatcgtcgggtttcccaccaaactgtttatccgtctacctcgctaccgctgcaccaaccccacatgtaagcaaaagtatttccaagcagaactaagctgcgctgaccacggtaaaaaggtcacccaccgggtcacccgctggattttacaacgccttgctattgaccggatgagtgttcacgcaaccgcgaaagcacttgggctagggtgggatttaacctgccaactagccctcgatatgtgccgtgagctggtctataacgatcctcaccatcttgatggagtgtatgtcattggggtggatgagcataagtggtcacataatagggctaagcatggtgatgggtttgtcaccgtgattgtcgatatgaccgggcatcggtatgactcacggtgtcctgcccggttattagatgtcgtcccaggtcgtagtgctgatgctttacggtcctggcttggctcccgcggtgaacagttccgcaatcagatacggatcgtgtccatggatggattccaaggctacgccacagcaagtaaagaactcattccttctgctcgtcgcgtgatggatccattccatgttgtgcggcttgctggtgacaagctcaccgcctgccggcaacgcctccagcgggagaaataccagcgtcgtggtttaagccaggatccgttgtataaaaaccggaagaccttgttgaccacgcacaagtggttgagtcctcgtcagcaagaaagcttggagcagttgtgggcgtatgacaaagactacggggcgttaaagcttgcgtggcttgcgtatcaggcgattattgattgttatcagatgggtaataagcgtgaagcgaagaagaaaatgcggaccattattgatcagcttcgggtgttgaaggggccgaataaggaactcgcgcagttgggtcgtagtttgtttaaacgacttggtgatgtgttggcgtatttcgatgttggtgtctccaacggtccggtcgaagcgatcaacggacggttggagcatttgcgtgggattgctctaggtttccgtaatttgaaccactacattctgcggtgccttatccattcagggcagttggtccataagatcaatgcactctaa

SEQ ID NO: 75 - DNA, 31 bp, synthetic construct
  source 1..31: mol_type = other DNA
ttcgagctcggtacccatgaagtctaccggc

SEQ ID NO: 76 - DNA, 30 bp, synthetic construct
  source 1..30: mol_type = other DNA
gacatgaagcgccgacatctaataaccggg

SEQ ID NO: 77 - DNA, 32 bp, synthetic construct
  source 1..32: mol_type = other DNA
ccgacgaggcctaagaactcattccttctgct

SEQ ID NO: 78 - DNA, 31 bp, synthetic construct
  source 1..31: mol_type = other DNA
ctctagaggatccccttagagtgcattgatc

SEQ ID NO: 79 - DNA, 30 bp, synthetic construct
  source 1..30: mol_type = other DNA
ccggttattagatgtcggcgcttcatgtca

SEQ ID NO: 80 - DNA, 25 bp, synthetic construct
  source 1..25: mol_type = other DNA
ggatgtttctctagatgcgggcgat

SEQ ID NO: 81 - DNA, 29 bp, synthetic construct
  source 1..29: mol_type = other DNA
gcccgcatctagagaaacatcccagcgct

SEQ ID NO: 82 - DNA, 29 bp, synthetic construct
  source 1..29: mol_type = other DNA
agaaggaatgagttcttaggcctcgtcgg

SEQ ID NO: 83 - DNA, 19 bp, synthetic construct
  source 1..19: mol_type = other DNA
ctttcagctttccctcccg

SEQ ID NO: 84 - DNA, 17 bp, synthetic construct
  source 1..17: mol_type = other DNA
gctgtacttttagtaca

SEQ ID NO: 85 - DNA, 5802 bp, synthetic construct
  source 1..5802: mol_type = other DNA
gttcgcttgctgtccataaaaccgcccagtctagctatcgccatgtaagcccactgcaagctacctgctttctctttgcgcttgcgttttcccttgtccagatagcccagtagctgacattcatccggggtcagcaccgtttctgcggactggctttctacgtgttccgcttcctttagcagcccttgcgccctgagtgcttgcggcagcgtgaagctagcttttatcgccattcgccattcaggctgcgcaactgttgggaagggcgatcggtgcgggcctcttcgctattacgccagctggcgaaagggggatgtgctgcaaggcgattaagttgggtaacgccagggttttcccagtcacgacgttgtaaaacgacggccagtgaattcgagctcggtacccggggatcctctagagtcgacctgcaggcatgcaagcttggcgtaatcatggtcatagctgtttcctgtgtgaaattgttatccgctcacaattccacacaacatacgagccggaagcataaagtgtaaagcctggggtgcctaatgagtgagctaactcacattaattgcgttgcgctcactgcccgctttccagtcgggaaacctgtcgtgccagctgcattaatgaatcggccaacgcgcggggagaggcggtttgcgtattgggcgctcttccgcttcctcgctcactgactcgctgcgctcggtcgttcggctgcggcgagcggtatcagctcactcaaaggcggtaatacggttatccacagaatcaggggataacgcaggaaagaacatgtgagcaaaaggccagcaaaaggccaggaaccgtaaaaaggccgcgttgctggcgtttttccataggctccgcccccctgacgagcatcacaaaaatcgacgctcaagtcagaggtggcgaaacccgacaggactataaagataccaggcgtttccccctggaagctccctcgtgcgctctcctgttccgaccctgccgcttaccggatacctgtccgcctttctcccttcgggaagcgtggcgctttctcaatgctcacgctgtaggtatctcagttcggtgtaggtcgttcgctccaagctgggctgtgtgcacgaaccccccgttcagcccgaccgctgcgccttatccggtaactatcgtcttgagtccaacccggtaagacacgacttatcgccactggcagcagccactggtaacaggattagcagagcgaggtatgtaggcggtgctacagagttcttgaagtggtggcctaactacggctacactagaaggacagtatttggtatctgcgctctgctgaagccagttaccttcggaaaaagagttggtagctcttgatccggcaaacaaaccaccgctggtagcggtggtttttttgtttgcaagcagcagattacgcgcagaaaaaaaggatctcaagaagatcctttgatcttttctacggggtctgacgctcagtggaacgaaaactcacgttaagggattttggtcatgagattatcaaaaaggatcttcacctagatccttttggggtgggcgaagaactccagcatgagatccccgcgctggaggatcatccagccctgatagaaacagaagccactggagcacctcaaaaacaccatcatacactaaatcagtaagttggcagcatcacccgacgcactttgcgccgaataaatacctgtgacggaagatcacttcgcagaataaataaatcctggtgtccctgttgataccgggaagccctgggccaacttttggcgaaaatgagacgttgatcggcacgtaagaggttccaactttcaccataatgaaataagatcactaccgggcgtattttttgagttatcgagattttcaggagctgatagaaacagaagccactggagcacctcaaaaacaccatcatacactaaatcagtaagttggcagcatcacccgacgcactttgcgccgaataaatacctgtgacggaagatcacttcgcagaataaataaatcctggtgtccctgttgataccgggaagccctgggccaacttttggcgaaaatgagacgttgatcggcacgtaagaggttccaactttcaccataatgaaataagatcactaccgggcgtattttttgagttatcgagattttcaggagctctttggcatcgtctctcgcctgtcccctcagttcagtaatttcctgcatttgcctgtttccagtcggtagatattccacaaaacagcagggaagcagcgcttttccgctgcataaccctgcttcggggtcattatagcgattttttcggtatatccatcctttttcgcacgatatacaggattttgccaaagggttcgtgtagactttccttggtgtatccaacggcgtcagccgggcaggataggtgaagtaggcccacccgcgagcgggtgttccttcttcactgtcccttattcgcacctggcggtgctcaacgggaatcctgctctgcgaggctggccggctaccgccggcgtaacagatgagggcaagcggatggctgatgaaaccaagccaaccaggaagggcagcccacctatcaaggtgtactgccttccagacgaacgaagagcgattgaggaaaaggcggcggcggccggcatgagcctgtcggcctacctgctggccgtcggccagggctacaaaatcacgggcgtcgtggactatgagcacgtccgcgagggcgtcccggaaaacgattccgaagcccaacctttcatagaaggcggcggtggaatcgaaatctcgtgatggcaggttgggcgtcgcttggtcggtcatttcgaaaaaggttaggaatacggttagccatttgcctgcttttatatagttcatatgggattcacctttatgttgataagaaataaaagaaaatgccaataggatatcggcattttcttttgcgtttttatttgttaactgttaattgtccttgttcaaggatgctgtctttgacaacagatgttttcttgcctttgatgttcagcaggaagctcggcgcaaacgttgattgtttgtctgcgtagaatcctctgtttgtcatatagcttgtaatcacgacattgtttcctttcgcttgaggtacagcgaagtgtgagtaagtaaaggttacatcgttaggcggatcaagatccatttttaacacaaggccagttttgttcagcggcttgtatgggccagttaaagaattagaaacataaccaagcatgtaaatatcgttagacgtaatgccgtcaatcgtcatttttgatccgcgggagtcagtgaacaggtaccatttgccgttcattttaaagacgttcgcgcgttcaatttcatctgttactgtgttagatgcaatcagcggtttcatcacttttttcagtgtgtaatcatcgtttagctcaatcataccgagagcgccgtttgctaactcagccgtgcgttttttatcgctttgcagaagtttttgactttcttgacggaagaatgatgtgcttttgccatagtatgctttgttaaataaagattcttcgccttggtagccatcttcagttccagtgtttgcttcaaatactaagtatttgtggcctttatcttctacgtagtgaggatctctcagcgtatggttgtcgcctgagctgtagttgccttcatcgatgaactgctgtacattttgatacgtttttccgtcaccgtcaaagattgatttataatcctctacaccgttgatgttcaaagagctgtctgatgctgatacgttaacttgtgcagttgtcagtgtttgtttgccgtaatgtttaccggagaaatcagtgtagaataaacggatttttccgtcagatgtaaatgtggctgaacctgaccattcttgtgtttggtcttttaggatagaatcatttgcatcgaatttgtcgctgtctttaaagacgcggccagcgtttttccagctgtcaatagaagtttcgccgactttttgatagaacatgtaaatcgatgtgtcatccgcatttttaggatctccggctaatgcaaagacgatgtggtagccgtgatagtttgcgacagtgccgtcagcgttttgtaatggccagctgtcccaaacgtccaggccttttgcagaagagatatttttaattgtggacgaatcaaattcagaaacttgatatttttcatttttttgctgttcagggatttgcagcatatcatggcgtgtaatatgggaaatgccgtatgtttccttatatggcttttggttcgtttctttcgcaaacgcttgagttgcgcctcctgccagcagtgcggtagtaaaggttaatactgttgcttgttttgcaaactttttgatgttcatcgttcatgtctccttttttatgtactgtgttagcggtctgcttcttccagccctcctgtttgaagatggcaagttagttacgcacaataaaaaaagacctaaaatatgtaaggggtgacgccaaagtatacactttgccctttacacattttaggtcttgcctgctttatcagtaacaaacccgcgcgatttacttttcgacctcattctattagactctcgtttggattgcaactggtctattttcctcttttgtttgatagaaaatcataaaaggatttgcagactacgggcctaaagaactaaaaaatctatctgtttcttttcattctctgtattttttatagtttctgttgcatgggcataaagttgcctttttaatcacaattcagaaaatatcataatatctcatttcactaaataatagtgaacggcaggtatatgtgatgggttaaaaaggatcaccccagagtcccgctcagaagaactcgtcaagaaggcgatagaaggcgatgcgctgcgaatcgggagcggcgataccgtaaagcacgaggaagcggtcagcccattcgccgccaagctcttcagcaatatcacgggtagccaacgctatgtcctgatagcggtccgccacacccagccggccacagtcgatgaatccagaaaagcggccattttccaccatgatattcggcaagcaggcatcgccatgggtcacgacgagatcctcgccgtcgggcatccgcgccttgagcctggcgaacagttcggctggcgcgagcccctgatgctcttcgtccagatcatcctgatcgacaagaccggcttccatccgagtacgtgctcgctcgatgcgatgtttcgcttggtggtcgaatgggcaggtagccggatcaagcgtatgcagccgccgcattgcatcagccatgatggatactttctcggcaggagcaaggtgagatgacaggagatcctgccccggcacttcgcccaatagcagccagtcccttcccgcttcagtgacaacgtcgagacagctgcgcaaggaacgcccgtcgtggccagccacgatagccgcgctgcctcgtcttggagttcattcagggcaccggacaggtcggtcttgacaaaaagaaccgggcgcccctgcgctgacagccggaacacggcggcatcagagcagccgattgtctgttgtgcccagtcatagccgaatagcctctccacccaagcggccggagaacctgcgtgcaatccatcttgttcaatcatgcgaaacgatcctcatcctgtctcttgatcagatcttgatcccctgcgccatcagatccttggcggcaagaaagccatccagtttactttgcagggcttcccaaccttaccagagggcgccccagctggcaattccg